European Patent Specification EP 4 452 831 B1, published March 11, 2026. Title: Colorimetric Sensing with Reconfigurable Chiral Plasmonic Structures and a method for detecting analytes in samples using the same. Applicant: Aalto University Foundation sr. The sequence listing filed with the application follows.

SEQUENCE LISTING (20 sequences)

SEQ ID NO: 1 - DNA, 64 bp, synthetic construct
  source 1..64: mol_type = other DNA
ataccaaatcgcctatgttacctttgaatcaagagaaatcaatctccgccactacactcaactc

SEQ ID NO: 2 - DNA, 50 bp, synthetic construct
  source 1..50: mol_type = other DNA
tgagagttcgtaaaacaggaagcattaatgagttgagtgtagtggcggag

SEQ ID NO: 3 - DNA, 70 bp, synthetic construct
  source 1..70: mol_type = other DNA
ataccaaatcgcctatgttacctttgaatcaagagaaatcaatctccgccactacactcaactcaaatac

SEQ ID NO: 4 - DNA, 36 bp, synthetic construct
  source 1..36: mol_type = other DNA
gatgttgcttggtaatagttgagtgtagtggcggag

SEQ ID NO: 5 - DNA, 30 bp, synthetic construct
  source 1..30: mol_type = other DNA
gatgttgcttggtaatgtgtagtggcggag

SEQ ID NO: 6 - DNA, 44 bp, synthetic construct
  source 1..44: mol_type = other DNA
tgagagttcgtaaaacaggaagcattaatttaccaagcaacatc

SEQ ID NO: 7 - DNA, 35 bp, synthetic construct
  source 1..35: mol_type = other DNA
cgtaacaaagctggctggctgaccttcaagaggac

SEQ ID NO: 8 - DNA, 45 bp, synthetic construct
  source 1..45: mol_type = other DNA
ataccaaatcgcctatgttacctttgaatcaagagaaatcaattt

SEQ ID NO: 9 - DNA, 31 bp, synthetic construct
  source 1..31: mol_type = other DNA
tgagagttcgtaaaacaggaagcattaattt

SEQ ID NO: 10 - DNA, 42 bp, synthetic construct
  source 1..42: mol_type = other DNA
attgcccaagacttgtgtgttgagttgagtgtagtggcggag

SEQ ID NO: 11 - DNA, 43 bp, synthetic construct
  source 1..43: mol_type = other DNA
tgagagttcgtaaaacaggaagcattaattcacacaagtcttg

SEQ ID NO: 12 - DNA, 31 bp, synthetic construct
  source 1..31: mol_type = other DNA
cacacaagtcttgggcaatttgcttcaatgc

SEQ ID NO: 13 - DNA, 25 bp, synthetic construct
  source 1..25: mol_type = other DNA
gcattgaagcaaattgcccaagact

SEQ ID NO: 14 - DNA, 64 bp, synthetic construct
  source 1..64: mol_type = other DNA
ataccaaatcgcctatgttacctttgaatcaagagaaatcaatgaacctcactacagtcaactc

SEQ ID NO: 15 - DNA, 36 bp, synthetic construct
  source 1..36: mol_type = other DNA
tcccccaggtcgcgtgagttgactgtagtgaggttc

SEQ ID NO: 16 - DNA, 61 bp, synthetic construct
  source 1..61: mol_type = other DNA
tgagagttcgtaaaacaggaagcattaattcgcgacctgggggagtattgcggaggaaggt

SEQ ID NO: 17 - DNA, 28 bp, synthetic construct
  source 1..28: mol_type = other DNA
gcttcaatgccacttgtgtcccccaggt

SEQ ID NO: 18 - DNA, 31 bp, synthetic construct
  source 1..31: mol_type = other DNA
cgcgacctgggggagtattgcggaggaaggt

SEQ ID NO: 19 - DNA, 24 bp, synthetic construct
  source 1..24: mol_type = other DNA
gggggacacaagtggcattgaagc

SEQ ID NO: 20 - DNA, 16 bp, synthetic construct
  source 1..16: mol_type = other DNA
tttttttttttttttt